European Patent Application EP 4 273 161 A1, published November 8, 2023. Title: PROTEIN CONTAINING HETERODIMER ANTIBODY FC, AND PREPARATION METHOD THEREFOR. Applicant: Innovent Biologics (Suzhou) Co., Ltd. The sequence listing filed with the application follows.

SEQUENCE LISTING (49 sequences)

SEQ ID NO: 1 - protein, 450 aa, Artificial
  Synthetic polypeptide
QVQLVQSGAEVKKPGSSVKVSCKASGGTFSSYAISWVRQAPGQGLEWMGLIIPMFDTAGYAQKFQGRVAITVDESTSTAYMELSSLRSEDTAVYYCARAEHSSTGTFDYWGQGTLVTVSSASTKGPSVFPLAPSSKSTSGGTAALGCLVKDYFPEPVTVSWNSGALTSGVHTFPAVLQSSGLYSLSSVVTVPSSSLGTQTYICNVNHKPSNTKVDKKVEPKSCDKTHTCPPCPAPEAAGGPSVFLFPPKPKDTLMISRTPEVTCVVVDVSHEDPEVKFNWYVDGVEVHNAKTKPREEQYNSTYRVVSVLTVLHQDWLNGKEYKCKVSNKALPAPIEKTISKAKGQPREPQVYVLPPSRDNLTKNQVRLTCLVKGFYPSDIAVEWESNGQPENNYKTTPPVLKSDGSFFLYSKLTVDKSRWQQGNVFSCSVMHEALHNHYTQKSLSLSPGK

SEQ ID NO: 2 - protein, 366 aa, Artificial
  Synthetic polypeptide
APASSSTKKTQLQLEHLLLDLQMILNGINNYKNPELEEMLTAKFYMPKKATELKHLQCLEEELKPLEEVLNLAGDASIHDLISNINVIVLELKGSETTFMCEYADETATIVEFLNRWITFSQSIISTLTGGGGSGGGGSDKTHTCPPCPAPEAAGGPSVFLFPPKPKDTLMISRTPEVTCVVVDVSHEDPEVKFNWYVDGVEVHNAKTKPREEQYNSTYRVVSVLTVLHQDWLNGKEYKCKVSNKALPAPIEKTISKAKGQPREPDVTVLPPSRDELTKNQVSLTCLVSGFYPSDIAVEWESNGQPENNYKTTPPVLDSDGSFFLYSDLTVDKSRWQQGNVFSCSVMHEALHNHYTQKSLSLSPGK

SEQ ID NO: 3 - protein, 450 aa, Artificial
  Synthetic polypeptide
QVQLVQSGAEVKKPGSSVKVSCKASGGTFSSYAISWVRQAPGQGLEWMGLIIPMFDTAGYAQKFQGRVAITVDESTSTAYMELSSLRSEDTAVYYCARAEHSSTGTFDYWGQGTLVTVSSASTKGPSVFPLAPSSKSTSGGTAALGCLVKDYFPEPVTVSWNSGALTSGVHTFPAVLQSSGLYSLSSVVTVPSSSLGTQTYICNVNHKPSNTKVDKKVEPKSCDKTHTCPPCPAPEAAGGPSVFLFPPKPKDTLMISRTPEVTCVVVDVSHEDPEVKFNWYVDGVEVHNAKTKPREEQYNSTYRVVSVLTVLHQDWLNGKEYKCKVSNKALPAPIEKTISKAKGQPREPQVYTLPPSRDELTKNQVSLTCLVKGFYPSDIAVEWESNGQPENNYKTTPPVLDSDGSFFLYSELRVDKSRWQQGNVFSCSVMHEALHNHYTQKSLSLSPGK

SEQ ID NO: 4 - protein, 366 aa, Artificial
  Synthetic polypeptide
APASSSTKKTQLQLEHLLLDLQMILNGINNYKNPELEEMLTAKFYMPKKATELKHLQCLEEELKPLEEVLNLAGDASIHDLISNINVIVLELKGSETTFMCEYADETATIVEFLNRWITFSQSIISTLTGGGGSGGGGSDKTHTCPPCPAPEAAGGPSVFLFPPKPKDTLMISRTPEVTCVVVDVSHEDPEVKFNWYVDGVEVHNAKTKPREEQYNSTYRVVSVLTVLHQDWLNGKEYKCKVSNKALPAPIEKTISKAKGQPREPQVYTLPPSRDELTKNQVSLTCLVTGFYPSDIAVEWESNGQPENNYKTTPPVLKSDGSFFLYSKLTVDKSRWQQGNVFSCSVMHEALHNHYTQKSLSLSPGK

SEQ ID NO: 5 - protein, 451 aa, Artificial
  Synthetic polypeptide
QVQLQQPGAELVKPGASVKMSCKASGYTFTSYNMHWVKQTPGRGLEWIGAIYPGNGDTSYNQKFKGKATLTADKSSSTAYMQLSSLTSEDSAVYYCARSTYYGGDWYFNVWGAGTTVTVSAASTKGPSVFPLAPSSKSTSGGTAALGCLVKDYFPEPVTVSWNSGALTSGVHTFPAVLQSSGLYSLSSVVTVPSSSLGTQTYICNVNHKPSNTKVDKKVEPKSCDKTHTCPPCPAPEAAGGPSVFLFPPKPKDTLMISRTPEVTCVVVDVSHEDPEVKFNWYVDGVEVHNAKTKPREEQYNSTYRVVSVLTVLHQDWLNGKEYKCKVSNKALPAPIEKTISKAKGQPREPDVTVLPPSRDELTKNQVSLTCLVSGFYPSDIAVEWESNGQPENNYKTTPPVLDSDGSFFLYSDLTVDKSRWQQGNVFSCSVMHEALHNHYTQKSLSLSPGK

SEQ ID NO: 6 - protein, 450 aa, Artificial
  Synthetic polypeptide
QVQLVQSGAEVKKPGSSVKVSCKASGGTFSSYAISWVRQAPGQGLEWMGLIIPMFDTAGYAQKFQGRVAITVDESTSTAYMELSSLRSEDTAVYYCARAEHSSTGTFDYWGQGTLVTVSSASTKGPSVFPLAPSSKSTSGGTAALGCLVKDYFPEPVTVSWNSGALTSGVHTFPAVLQSSGLYSLSSVVTVPSSSLGTQTYICNVNHKPSNTKVDKKVEPKSCDKTHTCPPCPAPEAAGGPSVFLFPPKPKDTLMISRTPEVTCVVVDVSHEDPEVKFNWYVDGVEVHNAKTKPREEQYNSTYRVVSVLTVLHQDWLNGKEYKCKVSNKALPAPIEKTISKAKGQPREPQVYTLPPSRDNLTKNQVRLTCLVKGFYPSDIAVEWESNGQPENNYKTTPPVLKSDGSFFLYSKLTVDKSRWQQGNVFSCSVMHEALHNHYTQKSLSLSPGK

SEQ ID NO: 7 - protein, 450 aa, Artificial
  Synthetic polypeptide
QVQLVQSGAEVKKPGSSVKVSCKASGGTFSSYAISWVRQAPGQGLEWMGLIIPMFDTAGYAQKFQGRVAITVDESTSTAYMELSSLRSEDTAVYYCARAEHSSTGTFDYWGQGTLVTVSSASTKGPSVFPLAPSSKSTSGGTAALGCLVKDYFPEPVTVSWNSGALTSGVHTFPAVLQSSGLYSLSSVVTVPSSSLGTQTYICNVNHKPSNTKVDKKVEPKSCDKTHTCPPCPAPEAAGGPSVFLFPPKPKDTLMISRTPEVTCVVVDVSHEDPEVKFNWYVDGVEVHNAKTKPREEQYNSTYRVVSVLTVLHQDWLNGKEYKCKVSNKALPAPIEKTISKAKGQPREPQVYTLPPSRDELTKNQVRLTCLVKGFYPSDIAVEWESNGQPENNYKTTPPVLKSDGSFFLYSKLTVDKSRWQQGNVFSCSVMHEALHNHYTQKSLSLSPGK

SEQ ID NO: 8 - protein, 366 aa, Artificial
  Synthetic polypeptide
APASSSTKKTQLQLEHLLLDLQMILNGINNYKNPELEEMLTAKFYMPKKATELKHLQCLEEELKPLEEVLNLAGDASIHDLISNINVIVLELKGSETTFMCEYADETATIVEFLNRWITFSQSIISTLTGGGGSGGGGSDKTHTCPPCPAPEAAGGPSVFLFPPKPKDTLMISRTPEVTCVVVDVSHEDPEVKFNWYVDGVEVHNAKTKPREEQYNSTYRVVSVLTVLHQDWLNGKEYKCKVSNKALPAPIEKTISKAKGQPREPDVTTLPPSRDELTKNQVSLTCLVSGFYPSDIAVEWESNGQPENNYKTTPPVLDSDGSFFLYSDLTVDKSRWQQGNVFSCSVMHEALHNHYTQKSLSLSPGK

SEQ ID NO: 9 - protein, 366 aa, Artificial
  Synthetic polypeptide
APASSSTKKTQLQLEHLLLDLQMILNGINNYKNPELEEMLTAKFYMPKKATELKHLQCLEEELKPLEEVLNLAGDASIHDLISNINVIVLELKGSETTFMCEYADETATIVEFLNRWITFSQSIISTLTGGGGSGGGGSDKTHTCPPCPAPEAAGGPSVFLFPPKPKDTLMISRTPEVTCVVVDVSHEDPEVKFNWYVDGVEVHNAKTKPREEQYNSTYRVVSVLTVLHQDWLNGKEYKCKVSNKALPAPIEKTISKAKGQPREPQVTTLPPSRDELTKNQVSLTCLVSGFYPSDIAVEWESNGQPENNYKTTPPVLDSDGSFFLYSDLTVDKSRWQQGNVFSCSVMHEALHNHYTQKSLSLSPGK

SEQ ID NO: 10 - protein, 451 aa, Artificial
  Synthetic polypeptide
QVQLQQPGAELVKPGASVKMSCKASGYTFTSYNMHWVKQTPGRGLEWIGAIYPGNGDTSYNQKFKGKATLTADKSSSTAYMQLSSLTSEDSAVYYCARSTYYGGDWYFNVWGAGTTVTVSAASTKGPSVFPLAPSSKSTSGGTAALGCLVKDYFPEPVTVSWNSGALTSGVHTFPAVLQSSGLYSLSSVVTVPSSSLGTQTYICNVNHKPSNTKVDKKVEPKSCDKTHTCPPCPAPEAAGGPSVFLFPPKPKDTLMISRTPEVTCVVVDVSHEDPEVKFNWYVDGVEVHNAKTKPREEQYNSTYRVVSVLTVLHQDWLNGKEYKCKVSNKALPAPIEKTISKAKGQPREPQVYTLPPSRDELTKNQVRLTCLVKGFYPSDIAVEWESNGQPENNYKTTPPVLKSDGSFFLYSKLTVDKSRWQQGNVFSCSVMHEALHNHYTQKSLSLSPGK

SEQ ID NO: 11 - protein, 445 aa, Artificial
  Synthetic polypeptide
QVQLVQSGAEVKKPGASVKVSCKASGYTFTDYEMHWVRQAPGQGLEWMGALDPKTGDTAYSQKFKGRVTLTADKSTSTAYMELSSLTSEDTAVYYCTRFYSYTYWGQGTLVTVSSASTKGPSVFPLAPSSKSTSGGTAALGCLVKDYFPEPVTVSWNSGALTSGVHTFPAVLQSSGLYSLSSVVTVPSSSLGTQTYICNVNHKPSNTKVDKKVEPKSCDKTHTCPPCPAPEAAGGPSVFLFPPKPKDTLMISRTPEVTCVVVDVSHEDPEVKFNWYVDGVEVHNAKTKPREEQYNSTYRVVSVLTVLHQDWLNGKEYKCKVSNKALPAPIEKTISKAKGQPREPQVYTLPPSRDELTKNQVRLTCLVKGFYPSDIAVEWESNGQPENNYKTTPPVLKSDGSFFLYSKLTVDKSRWQQGNVFSCSVMHEALHNHYTQKSLSLSPGK

SEQ ID NO: 12 - protein, 450 aa, Artificial
  Synthetic polypeptide
QVQLVQSGAEVKKPGSSVKVSCKASGGTFSSYAISWVRQAPGQGLEWMGLIIPMFDTAGYAQKFQGRVAITVDESTSTAYMELSSLRSEDTAVYYCARAEHSSTGTFDYWGQGTLVTVSSASTKGPSVFPLAPSSKSTSGGTAALGCLVKDYFPEPVTVSWNSGALTSGVHTFPAVLQSSGLYSLSSVVTVPSSSLGTQTYICNVNHKPSNTKVDKKVEPKSCDKTHTCPPCPAPEAAGGPSVFLFPPKPKDTLMISRTPEVTCVVVDVSHEDPEVKFNWYVDGVEVHNAKTKPREEQYNSTYRVVSVLTVLHQDWLNGKEYKCKVSNKALPAPIEKTISKAKGQPREPQVTTLPPSRDELTKNQVSLTCLVSGFYPSDIAVEWESNGQPENNYKTTPPVLDSDGSFFLYSDLTVDKSRWQQGNVFSCSVMHEALHNHYTQKSLSLSPGK

SEQ ID NO: 13 - protein, 364 aa, Artificial
  Synthetic polypeptide
QVQLQESGGGLVQPGGSLRLSCAASAYTISRNSMGWFRQAPGKGLEGVAAIESDGSTSYSDSVKGRFTISLDNSKNTLYLEMNSLRAEDTAVYYCAAPKVGLGPRTALGHLAFMTLPALNYWGQGTLVTVSSEPKSSDKTHTCPPCPAPEAAGGPSVFLFPPKPKDTLMISRTPEVTCVVVDVSHEDPEVKFNWYVDGVEVHNAKTKPREEQYNSTYRVVSVLTVLHQDWLNGKEYKCKVSNKALPAPIEKTISKAKGQPREPQVTTLPPSRDELTKNQVSLTCLVSGFYPSDIAVEWESNGQPENNYKTTPPVLDSDGSFFLYSDLTVDKSRWQQGNVFSCSVMHEALHNHYTQKSLSLSPGK

SEQ ID NO: 14 - protein, 451 aa, Artificial
  Synthetic polypeptide
QVQLQQPGAELVKPGASVKMSCKASGYTFTSYNMHWVKQTPGRGLEWIGAIYPGNGDTSYNQKFKGKATLTADKSSSTAYMQLSSLTSEDSAVYYCARSTYYGGDWYFNVWGAGTTVTVSAASTKGPSVFPLAPSSKSTSGGTAALGCLVKDYFPEPVTVSWNSGALTSGVHTFPAVLQSSGLYSLSSVVTVPSSSLGTQTYICNVNHKPSNTKVDKKVEPKSCDKTHTCPPCPAPEAAGGPSVFLFPPKPKDTLMISRTPEVTCVVVDVSHEDPEVKFNWYVDGVEVHNAKTKPREEQYNSTYRVVSVLTVLHQDWLNGKEYKCKVSNKALPAPIEKTISKAKGQPREPQVTTLPPSRDELTKNQVSLTCLVSGFYPSDIAVEWESNGQPENNYKTTPPVLDSDGSFFLYSDLTVDKSRWQQGNVFSCSVMHEALHNHYTQKSLSLSPGK

SEQ ID NO: 15 - protein, 464 aa, Artificial
  Synthetic polypeptide
DIQMTQSPSSVSASVGDRVTITCRASQGISRWLAWYQQKPGKAPKLLIYAASSLQSGVPSRFSGSGSGTDFTLTISSLQPEDFATYYCQQTVSFPITFGGGTKVEIKGGGGSGGGGSGGGGSQVQLQESGPGLVKPSETLSLTCTVSGGSIEHYYWSWIRQPPGKGLEWIGYIYYSGSTNYNPSLKSRVTISVDTSKNQFSLKLSSVTAADTAVYYCARGKTGSAAWGQGTLVTVSSDKTHTCPPCPAPEAAGGPSVFLFPPKPKDTLMISRTPEVTCVVVDVSHEDPEVKFNWYVDGVEVHNAKTKPREEQYNSTYRVVSVLTVLHQDWLNGKEYKCKVSNKALPAPIEKTISKAKGQPREPQVTTLPPSRDELTKNQVSLTCLVSGFYPSDIAVEWESNGQPENNYKTTPPVLDSDGSFFLYSDLTVDKSRWQQGNVFSCSVMHEALHNHYTQKSLSLSPGK

SEQ ID NO: 16 - protein, 450 aa, Artificial
  Synthetic polypeptide
EVQLVESGGGLVQPGGSLRLSCAASGFNIKDTYIHWVRQAPGKGLEWVARIYPTNGYTRYADSVKGRFTISADTSKNTAYLQMNSLRAEDTAVYYCSRWGGDGFYAMDYWGQGTLVTVSSASTKGPSVFPLAPSSKSTSGGTAALGCLVKDYFPEPVTVSWNSGALTSGVHTFPAVLQSSGLYSLSSVVTVPSSSLGTQTYICNVNHKPSNTKVDKKVEPKSCDKTHTCPPCPAPEAAGGPSVFLFPPKPKDTLMISRTPEVTCVVVDVSHEDPEVKFNWYVDGVEVHNAKTKPREEQYNSTYRVVSVLTVLHQDWLNGKEYKCKVSNKALPAPIEKTISKAKGQPREPQVYTLPPSRDELTKNQVRLTCLVKGFYPSDIAVEWESNGQPENNYKTTPPVLKSDGSFFLYSKLTVDKSRWQQGNVFSCSVMHEALHNHYTQKSLSLSPGK

SEQ ID NO: 17 - protein, 214 aa, Artificial
  Synthetic polypeptide
DIQMTQSPSSVSASVGDRVTITCRASQGISSWLAWYQQKPGKAPKLLISAASSLQSGVPSRFSGSGSGTDFTLTISSLQPEDFATYYCQQANHLPFTFGGGTKVEIKRTVAAPSVFIFPPSDEQLKSGTASVVCLLNNFYPREAKVQWKVDNALQSGNSQESVTEQDSKDSTYSLSSTLTLSKADYEKHKVYACEVTHQGLSSPVTKSFNRGEC

SEQ ID NO: 18 - protein, 214 aa, Artificial
  Synthetic polypeptide
DIQMTQSPSSLSASVGDRVTITCKASQDVSIGVAWYQQKPGKAPKLLIYSASYRYTGVPSRFSGSGSGTDFTLTISSLQPEDFATYYCQQYYIYPYTFGQGTKVEIKRTVAAPSVFIFPPSDEQLKSGTASVVCLLNNFYPREAKVQWKVDNALQSGNSQESVTEQDSKDSTYSLSSTLTLSKADYEKHKVYACEVTHQGLSSPVTKSFNRGEC

SEQ ID NO: 19 - protein, 213 aa, Artificial
  Synthetic polypeptide
QIVLSQSPAILSASPGEKVTMTCRASSSVSYIHWFQQKPGSSPKPWIYATSNLASGVPVRFSGSGSGTSYSLTISRVEAEDAATYYCQQWTSNPPTFGGGTKLEIKRTVAAPSVFIFPPSDEQLKSGTASVVCLLNNFYPREAKVQWKVDNALQSGNSQESVTEQDSKDSTYSLSSTLTLSKADYEKHKVYACEVTHQGLSSPVTKSFNRGEC

SEQ ID NO: 20 - protein, 219 aa, Artificial
  Synthetic polypeptide
DVVMTQSPLSLPVTPGEPASISCRSSQSLVHSNRNTYLHWYLQKPGQSPQLLIYKVSNRFSGVPDRFSGSGSGTDFTLKISRVEAEDVGVYYCSQNTHVPPTFGQGTKLEIKRTVAAPSVFIFPPSDEQLKSGTASVVCLLNNFYPREAKVQWKVDNALQSGNSQESVTEQDSKDSTYSLSSTLTLSKADYEKHKVYACEVTHQGLSSPVTKSFNRGEC

SEQ ID NO: 21 - protein, 120 aa, Artificial
  Synthetic polypeptide
QVQLVQSGAEVKKPGSSVKVSCKASGGTFSSYAISWVRQAPGQGLEWMGLIIPMFDTAGYAQKFQGRVAITVDESTSTAYMELSSLRSEDTAVYYCARAEHSSTGTFDYWGQGTLVTVSS

SEQ ID NO: 22 - protein, 98 aa, Artificial
  Synthetic polypeptide
ASTKGPSVFPLAPSSKSTSGGTAALGCLVKDYFPEPVTVSWNSGALTSGVHTFPAVLQSSGLYSLSSVVTVPSSSLGTQTYICNVNHKPSNTKVDKKV

SEQ ID NO: 23 - protein, 15 aa, Artificial
  Synthetic polypeptide
EPKSCDKTHTCPPCP

SEQ ID NO: 24 - protein, 110 aa, Artificial
  Synthetic polypeptide
APEAAGGPSVFLFPPKPKDTLMISRTPEVTCVVVDVSHEDPEVKFNWYVDGVEVHNAKTKPREEQYNSTYRVVSVLTVLHQDWLNGKEYKCKVSNKALPAPIEKTISKAK

SEQ ID NO: 25 - protein, 107 aa, Artificial
  Synthetic polypeptide
GQPREPQVYVLPPSRDNLTKNQVRLTCLVKGFYPSDIAVEWESNGQPENNYKTTPPVLKSDGSFFLYSKLTVDKSRWQQGNVFSCSVMHEALHNHYTQKSLSLSPGK

SEQ ID NO: 26 - protein, 129 aa, Artificial
  Synthetic polypeptide
APASSSTKKTQLQLEHLLLDLQMILNGINNYKNPELEEMLTAKFYMPKKATELKHLQCLEEELKPLEEVLNLAGDASIHDLISNINVIVLELKGSETTFMCEYADETATIVEFLNRWITFSQSIISTLT

SEQ ID NO: 27 - protein, 20 aa, Artificial
  Synthetic polypeptide
GGGGSGGGGSDKTHTCPPCP

SEQ ID NO: 28 - protein, 107 aa, Artificial
  Synthetic polypeptide
GQPREPDVTVLPPSRDELTKNQVSLTCLVSGFYPSDIAVEWESNGQPENNYKTTPPVLDSDGSFFLYSDLTVDKSRWQQGNVFSCSVMHEALHNHYTQKSLSLSPGK

SEQ ID NO: 29 - protein, 107 aa, Artificial
  Synthetic polypeptide
GQPREPQVYTLPPSRDELTKNQVSLTCLVKGFYPSDIAVEWESNGQPENNYKTTPPVLDSDGSFFLYSELRVDKSRWQQGNVFSCSVMHEALHNHYTQKSLSLSPGK

SEQ ID NO: 30 - protein, 107 aa, Artificial
  Synthetic polypeptide
GQPREPQVYTLPPSRDELTKNQVSLTCLVTGFYPSDIAVEWESNGQPENNYKTTPPVLKSDGSFFLYSKLTVDKSRWQQGNVFSCSVMHEALHNHYTQKSLSLSPGK

SEQ ID NO: 31 - protein, 121 aa, Artificial [sequence omitted]

SEQ ID NO: 32 - protein, 107 aa, Artificial
  Synthetic polypeptide
GQPREPQVYTLPPSRDNLTKNQVRLTCLVKGFYPSDIAVEWESNGQPENNYKTTPPVLKSDGSFFLYSKLTVDKSRWQQGNVFSCSVMHEALHNHYTQKSLSLSPGK

SEQ ID NO: 33 - protein, 107 aa, Artificial
  Synthetic polypeptide
GQPREPQVYTLPPSRDELTKNQVRLTCLVKGFYPSDIAVEWESNGQPENNYKTTPPVLKSDGSFFLYSKLTVDKSRWQQGNVFSCSVMHEALHNHYTQKSLSLSPGK

SEQ ID NO: 34 - protein, 107 aa, Artificial
  Synthetic polypeptide
GQPREPDVTTLPPSRDELTKNQVSLTCLVSGFYPSDIAVEWESNGQPENNYKTTPPVLDSDGSFFLYSDLTVDKSRWQQGNVFSCSVMHEALHNHYTQKSLSLSPGK

SEQ ID NO: 35 - protein, 107 aa, Artificial
  Synthetic polypeptide
GQPREPQVTTLPPSRDELTKNQVSLTCLVSGFYPSDIAVEWESNGQPENNYKTTPPVLDSDGSFFLYSDLTVDKSRWQQGNVFSCSVMHEALHNHYTQKSLSLSPGK

SEQ ID NO: 36 - protein, 115 aa, Artificial
  Synthetic polypeptide
QVQLVQSGAEVKKPGASVKVSCKASGYTFTDYEMHWVRQAPGQGLEWMGALDPKTGDTAYSQKFKGRVTLTADKSTSTAYMELSSLTSEDTAVYYCTRFYSYTYWGQGTLVTVSS

SEQ ID NO: 37 - protein, 132 aa, Artificial
  Synthetic polypeptide
QVQLQESGGGLVQPGGSLRLSCAASAYTISRNSMGWFRQAPGKGLEGVAAIESDGSTSYSDSVKGRFTISLDNSKNTLYLEMNSLRAEDTAVYYCAAPKVGLGPRTALGHLAFMTLPALNYWGQGTLVTVSS

SEQ ID NO: 38 - protein, 15 aa, Artificial
  Synthetic polypeptide
EPKSSDKTHTCPPCP

SEQ ID NO: 39 - protein, 237 aa, Artificial
  Synthetic polypeptide
DIQMTQSPSSVSASVGDRVTITCRASQGISRWLAWYQQKPGKAPKLLIYAASSLQSGVPSRFSGSGSGTDFTLTISSLQPEDFATYYCQQTVSFPITFGGGTKVEIKGGGGSGGGGSGGGGSQVQLQESGPGLVKPSETLSLTCTVSGGSIEHYYWSWIRQPPGKGLEWIGYIYYSGSTNYNPSLKSRVTISVDTSKNQFSLKLSSVTAADTAVYYCARGKTGSAAWGQGTLVTVSS

SEQ ID NO: 40 - protein, 10 aa, Artificial
  Synthetic polypeptide
DKTHTCPPCP

SEQ ID NO: 41 - protein, 120 aa, Artificial [sequence omitted]

SEQ ID NO: 42 - protein, 107 aa, Artificial
  Synthetic polypeptide
DIQMTQSPSSVSASVGDRVTITCRASQGISSWLAWYQQKPGKAPKLLISAASSLQSGVPSRFSGSGSGTDFTLTISSLQPEDFATYYCQQANHLPFTFGGGTKVEIK

SEQ ID NO: 43 - protein, 107 aa, Artificial [sequence omitted]

SEQ ID NO: 44 - protein, 107 aa, Artificial [sequence omitted]

SEQ ID NO: 45 - protein, 106 aa, Artificial [sequence omitted]

SEQ ID NO: 46 - protein, 112 aa, Artificial
  Synthetic polypeptide
DVVMTQSPLSLPVTPGEPASISCRSSQSLVHSNRNTYLHWYLQKPGQSPQLLIYKVSNRFSGVPDRFSGSGSGTDFTLKISRVEAEDVGVYYCSQNTHVPPTFGQGTKLEIK

SEQ ID NO: 47 - protein, 330 aa, Artificial [sequence omitted]

SEQ ID NO: 48 - protein, 227 aa, Artificial
  Synthetic polypeptide
DKTHTCPPCPAPELLGGPSVFLFPPKPKDTLMISRTPEVTCVVVDVSHEDPEVKFNWYVDGVEVHNAKTKPREEQYNSTYRVVSVLTVLHQDWLNGKEYKCKVSNKALPAPIEKTISKAKGQPREPQVYTLPPSRDELTKNQVSLTCLVKGFYPSDIAVEWESNGQPENNYKTTPPVLDSDGSFFLYSKLTVDKSRWQQGNVFSCSVMHEALHNHYTQKSLSLSPGK

SEQ ID NO: 49 - protein, 107 aa, Artificial
  Synthetic polypeptide
GQPREPQVYTLPPSRDELTKNQVSLTCLVKGFYPSDIAVEWESNGQPENNYKTTPPVLDSDGSFFLYSKLTVDKSRWQQGNVFSCSVMHEALHNHYTQKSLSLSPGK